European Patent Application EP 4 470 543 A1, published December 4, 2024. Title: Composition comprising RNA for transdermal administration and administration method of the same. Applicant: NanoCarrier Co.,Ltd. Application JP. The sequence listing filed with the application follows.

SEQUENCE LISTING (7 sequences)

SEQ ID NO: 1 - RNA, 24 nt, synthetic construct
  misc_feature 1..24: note = RNA 1 for double strand RNA
  source 1..24: mol_type = other RNA
ggtgtgtgtgtgtgtgtgtgtgtg

SEQ ID NO: 2 - DNA, 37 bp, synthetic construct
  misc_feature 1..37: note = DNA template
  source 1..37: mol_type = other DNA
acgactcactataggtgtgtgtgtgtgtgtgtgtgtg

SEQ ID NO: 3 - RNA, 43 nt, synthetic construct
  misc_feature 1..43: note = RNA 2 for double strand RNA
  source 1..43: mol_type = other RNA
ggttcaggatgtcccgcttcacacacacacacacacacacacc

SEQ ID NO: 4 - RNA, 43 nt, synthetic construct
  misc_feature 1..43: note = RNA 3 for double strand RNA
  source 1..43: mol_type = other RNA
gggcaggatggggtaccttcacacacacacacacacacacacc

SEQ ID NO: 5 - RNA, 43 nt, synthetic construct
  misc_feature 1..43: note = RNA 4 for double strand RNA
  source 1..43: mol_type = other RNA
gtcctcgtccttgaaggatcacacacacacacacacacacacc

SEQ ID NO: 6 - RNA, 43 nt, synthetic construct
  misc_feature 1..43: note = RNA 5 for double strand RNA
  source 1..43: mol_type = other RNA
gcttctcgaagttgatgtacacacacacacacacacacacacc

SEQ ID NO: 7 - RNA, 43 nt, synthetic construct
  misc_feature 1..43: note = RNA 6 for double strand RNA
  source 1..43: mol_type = other RNA
ggcgatgtgcttgatgcttcacacacacacacacacacacacc